European Patent Application EP 4 166 568 A1, published April 19, 2023. Title: Anti-human interleukin 23 monoclonal antibody and application thereof. Applicant: Qyuns therapeutics CO., Ltd. The sequence listing filed with the application follows.

SEQUENCE LISTING (12 sequences)

SEQ ID NO: 1 - protein, 5 aa, Artificial Sequence
  Description of Artificial Sequence: artificially synthesized sequence
NHEMS

SEQ ID NO: 2 - protein, 16 aa, Artificial Sequence
  Description of Artificial Sequence: artificially synthesized sequence
IITTSDTTYYATWAKG

SEQ ID NO: 3 - protein, 12 aa, Artificial Sequence
  Description of Artificial Sequence: artificially synthesized sequence
VDIVLLSVTSRI

SEQ ID NO: 4 - protein, 11 aa, Artificial Sequence
  Description of Artificial Sequence: artificially synthesized sequence
QASQSVSTYLS

SEQ ID NO: 5 - protein, 7 aa, Artificial Sequence
  Description of Artificial Sequence: artificially synthesized sequence
GASNLES

SEQ ID NO: 6 - protein, 10 aa, Artificial Sequence
  Description of Artificial Sequence: artificially synthesized sequence
QSGYVFAGLT

SEQ ID NO: 7 - protein, 120 aa, Artificial Sequence
  Description of Artificial Sequence: artificially synthesized sequence
EVQLVESGGGLVQPGGSLRLSCAASGFSLSNHEMSWVRQAPGKGLEWIGIITTSDTTYYATWAKGRFTISRDNSKNTLYLQMNSLRAEDTAVYYCARVDIVLLSVTSRIWGQGTLVTVSS

SEQ ID NO: 8 - protein, 108 aa, Artificial Sequence
  Description of Artificial Sequence: artificially synthesized sequence
DVVMTQSPSSLSASVGDRVTITCQASQSVSTYLSWYQQKPGKAPKLLIYGASNLESGVPSRFSGSGSGTDFTLTISSLQPEDFATYYCQSGYVFAGLTFGGGTKVEIK

SEQ ID NO: 9 - protein, 189 aa, Artificial Sequence
  Description of Artificial Sequence: artificially synthesized sequence
MLGSRAVMLLLLLPWTAQGRAVPGGSSPAWTQCQQLSQKLCTLAWSAHPLVGHMDLREEGDEETTNDVPHIQCGDGCDPQGLRDNSQFCLQRIHQGLIFYEKLLGSDIFTGEPSLLPDSPVGQLHASLLGLSQLLQPEGHHWETQQIPSLSPSQPWQRLLLRFKILRSLQAFVAVAARVFAHGAATLSP

SEQ ID NO: 10 - protein, 328 aa, Artificial Sequence
  Description of Artificial Sequence: artificially synthesized sequence
MCHQQLVISWFSLVFLASPLVAIWELKKDVYVVELDWYPDAPGEMVVLTCDTPEEDGITWTLDQSSEVLGSGKTLTIQVKEFGDAGQYTCHKGGEVLSHSLLLLHKKEDGIWSTDILKDQKEPKNKTFLRCEAKNYSGRFTCWWLTTISTDLTFSVKSSRGSSDPQGVTCGAATLSAERVRGDNKEYEYSVECQEDSACPAAEESLPIEVMVDAVHKLKYENYTSSFFIRDIIKPDPPKNLQLKPLKNSRQVEVSWEYPDTWSTPHSYFSLTFCVQVQGKSKREKKDRVFTDKTSATVICRKNASISVRAQDRYYSSSWSEWASVPCS

SEQ ID NO: 11 - protein, 450 aa, Artificial Sequence
  Description of Artificial Sequence: artificially synthesized sequence
EVQLVESGGGLVQPGGSLRLSCAASGFSLSNHEMSWVRQAPGKGLEWIGIITTSDTTYYATWAKGRFTISRDNSKNTLYLQMNSLRAEDTAVYYCARVDIVLLSVTSRIWGQGTLVTVSSASTKGPSVFPLAPSSKSTSGGTAALGCLVKDYFPEPVTVSWNSGALTSGVHTFPAVLQSSGLYSLSSVVTVPSSSLGTQTYICNVNHKPSNTKVDKKVEPKSCDKTHTCPPCPAPELLGGPSVFLFPPKPKDTLMISRTPEVTCVVVDVSHEDPEVKFNWYVDGVEVHNAKTKPREEQYNSTYRVVSVLTVLHQDWLNGKEYKCKVSNKALPAPIEKTISKAKGQPREPQVYTLPPSRDELTKNQVSLTCLVKGFYPSDIAVEWESNGQPENNYKTTPPVLDSDGSFFLYSKLTVDKSRWQQGNVFSCSVMHEALHNHYTQKSLSLSPGK

SEQ ID NO: 12 - protein, 215 aa, Artificial Sequence
  Description of Artificial Sequence: artificially synthesized sequence
DVVMTQSPSSLSASVGDRVTITCQASQSVSTYLSWYQQKPGKAPKLLIYGASNLESGVPSRFSGSGSGTDFTLTISSLQPEDFATYYCQSGYVFAGLTFGGGTKVEIKRTVAAPSVFIFPPSDEQLKSGTASVVCLLNNFYPREAKVQWKVDNALQSGNSQESVTEQDSKDSTYSLSSTLTLSKADYEKHKVYACEVTHQGLSSPVTKSFNRGEC